European Patent Application EP 4 667 468 A1, published December 24, 2025. Title: 一种抑制NLRP3的化合物及制备方法和应用. Applicant: 深圳众格生物科技有限公司. The sequence listing filed with the application follows.

SEQUENCE LISTING (1 sequence)

SEQ ID NO: 1 - protein, 1062 aa, synthetic construct
MHHHHHHGSGSDYKDDDDKENLYFQGMKMASTRCKLARYLEDLEDVDLKKFKMHLEDYPPQKGCIPLPRGQTEKADHVDLATLMIDFNGEEKAWAMAVWIFAAINRRDLYEKAKRDEPKWGSDNARVSNPTVICQEDSIEEEWMGLLEYLSRISICKMKKDYRKKYRKYVRSRFQCIEDRNARLGESVSLNKRYTRLRLIKEHRSQQEREQELLAIGKTKTCESPVSPIKMELLFDPDDEHSEPVHTVVFQGAAGIGKTILARKMMLDWASGTLYQDRFDYLFYIHCREVSLVTQRSLGDLIMSCCPDPNPPIHKIVRKPSRILFLMDGFDELQGAFDEHIGPLCTDWQKAERGDILLSSLIRKKLLPEASLLITTRPVALEKLQHLLDHPRHVEILGFSEAKRKEYFFKYFSDEAQARAAFSLIQENEVLFTMCFIPLVCWIVCTGLKQQMESGKSLAQTSKTTTAVYVFFLSSLLQPRGGSQEHGLCAHLWGLCSLAADGIWNQKILFEESDLRNHGLQKADVSAFLRMNLFQKEVDCEKFYSFIHMTFQEFFAAMYYLLEEEKEGRTNVPGSRLKLPSRDVTVLLENYGKFEKGYLIFVVRFLFGLVNQERTSYLEKKLSCKISQQIRLELLKWIEVKAKAKKLQIQPSQLELFYCLYEMQEEDFVQRAMDYFPKIEINLSTRMDHMVSSFCIENCHRVESLSLGFLHNMPKEEEEEEKEGRHLDMVQCVLPSSSHAACSHGLVNSHLTSSFCRGLFSVLSTSQSLTELDLSDNSLGDPGMRVLCETLQHPGCNIRRLWLGRCGLSHECCFDISLVLSSNQKLVELDLSDNALGDFGIRLLCVGLKHLLCNLKKLWLVSCCLTSACCQDLASVLSTSHSLTRLYVGENALGDSGVAILCEKAKNPQCNLQKLGLVNSGLTSVCCSALSSVLSTNQNLTHLYLRGNTLGDKGIKLLCEGLLHPDCKLQVLELDNCNLTSHCCWDLSTLLTSSQSLRKLSLGNNDLGDLGVMMFCEVLKQQSCLLQNLGLSEMYFNYETKSALETLQEEKPELTVVFEPSW